European Patent Application EP 4 529 929 A1, published April 2, 2025. Title: Isolated Nucleic Acid Molecule Comprising NKp30 Transmemebrane Domain and Chimeric Antigen Receptor Comprising the Same. Applicant: 沛爾生技醫藥股份有限公司. The sequence listing filed with the application follows.

SEQUENCE LISTING (97 sequences)

SEQ ID NO: 1 - protein, 242 aa, synthetic construct
  SITE 1..242: note = anti BCMA VHH1-GGGGS -VHH2
QVKLEESGGGLVQAGRSLRLSCAASEHTFSSHVMGWFRQAPGKERESVAVIGWRDISTSYADSVKGRFTISRDNAKKTLYLQMNSLKPEDTAVYYCAARRIDAADFDSWGQGTQVTVSSGGGGSEVQLVESGGGLVQAGGSLRLSCAASGRTFTMGWFRQAPGKEREFVAAISLSPTLAYYAESVKGRFTISRDNAKNTVVLQMNSLKPEDTALYYCAADRKSVMSIRPDYWGQGTQVTVSS

SEQ ID NO: 2 - protein, 119 aa, synthetic construct
  SITE 1..119: note = anti BCMA VHH1
QVKLEESGGGLVQAGRSLRLSCAASEHTFSSHVMGWFRQAPGKERESVAVIGWRDISTSYADSVKGRFTISRDNAKKTLYLQMNSLKPEDTAVYYCAARRIDAADFDSWGQGTQVTVSS

SEQ ID NO: 3 - protein, 118 aa, synthetic construct
  SITE 1..118: note = anti BCMA VHH2
EVQLVESGGGLVQAGGSLRLSCAASGRTFTMGWFRQAPGKEREFVAAISLSPTLAYYAESVKGRFTISRDNAKNTVVLQMNSLKPEDTALYYCAADRKSVMSIRPDYWGQGTQVTVSS

SEQ ID NO: 4 - protein, 9 aa, synthetic construct
  SITE 1..9: note = anti BCMA VHH1 CDRH1
HTFSSHVMG

SEQ ID NO: 5 - protein, 11 aa, synthetic construct
  SITE 1..11: note = anti BCMA VHH1 CDRH2
GWRDISTSYAD

SEQ ID NO: 6 - protein, 12 aa, synthetic construct
  SITE 1..12: note = anti BCMA VHH1 CDRH3
AARRIDAADFDS

SEQ ID NO: 7 - protein, 6 aa, synthetic construct
  SITE 1..6: note = anti BCMA VHH2 CDRH1
RTFTMG

SEQ ID NO: 8 - protein, 11 aa, synthetic construct
  SITE 1..11: note = anti BCMA VHH2 CDRH2
SLSPTLAYYAE

SEQ ID NO: 9 - protein, 14 aa, synthetic construct
  SITE 1..14: note = anti BCMA VHH2 CDRH3
AADRKSVMSIRPDY

SEQ ID NO: 10 - protein, 10 aa, synthetic construct
  SITE 1..10: note = anti CD19 antibody(FMC63) CDRH1
GVSLPDYGVS

SEQ ID NO: 11 - protein, 16 aa, synthetic construct
  SITE 1..16: note = anti CD19 antibody(FMC63) CDRH2
VIWGSETTYYNSALKS

SEQ ID NO: 12 - protein, 12 aa, synthetic construct
  SITE 1..12: note = anti CD19 antibody(FMC63) CDRH3
HYYYGGSYAMDY

SEQ ID NO: 13 - protein, 11 aa, synthetic construct
  SITE 1..11: note = anti CD19 antibody(FMC63) CDRL1
RASQDISKYLN

SEQ ID NO: 14 - protein, 7 aa, synthetic construct
  SITE 1..7: note = anti CD19 antibody(FMC63) CDRL2
SRLHSGV

SEQ ID NO: 15 - protein, 9 aa, synthetic construct
  SITE 1..9: note = anti CD19 antibody(FMC63) CDRL3
QQGNTLPYT

SEQ ID NO: 16 - protein, 242 aa, synthetic construct
  SITE 1..242: note = FMC63 scfv
DIQMTQTTSSLSASLGDRVTISCRASQDISKYLNWYQQKPDGTVKLLIYHTSRLHSGVPSRFSGSGSGTDYSLTISNLEQEDIATYFCQQGNTLPYTFGGGTKLEITGGGGSGGGGSGGGGSEVKLQESGPGLVAPSQSLSVTCTVSGVSLPDYGVSWIRQPPRKGLEWLGVIWGSETTYYNSALKSRLTIIKDNSKSQVFLKMNSLQTDDTAIYYCAKHYYYGGSYAMDYWGQGTSVTVSS

SEQ ID NO: 17 - protein, 5 aa, synthetic construct
  SITE 1..5: note = anti mesothelin antibody(SS1) CDRH1
GYTMN

SEQ ID NO: 18 - protein, 15 aa, synthetic construct
  SITE 1..15: note = anti mesothelin antibody(SS1) CDRH2
LITPYNGASSYNQKF

SEQ ID NO: 19 - protein, 10 aa, synthetic construct
  SITE 1..10: note = anti mesothelin antibody(SS1) CDRH3
GGYDGRGFDY

SEQ ID NO: 20 - protein, 10 aa, synthetic construct
  SITE 1..10: note = anti mesothelin antibody(SS1) CDRL1
SASSSVSYMH

SEQ ID NO: 21 - protein, 7 aa, synthetic construct
  SITE 1..7: note = anti mesothelin antibody(SS1) CDRL2
DTSKLAS

SEQ ID NO: 22 - protein, 9 aa, synthetic construct
  SITE 1..9: note = anti mesothelin antibody(SS1) CDRL3
QQWSKHPLT

SEQ ID NO: 23 - protein, 240 aa, synthetic construct
  SITE 1..240: note = SS1 scfv
QVQLQQSGPELEKPGASVKLSCKASGYSFTGYTMNWVKQSHGKSLEWIGLITPYNGASSYNQKFRGKATLTVDKSSSTAYMDLLSLTSEDSAVYFCARGGYDGRGFDYWGQGTTVTVSSGVGGSGGGGSGGGGSDIELTQSPAIMSASPGEKVTMTCSASSSVSYMHWYQQKSGTSPKRWIYDTSKLASGVPGRFSGSGSGNSYSLTISSVEAEDDATYYCQQWSKHPLTFGAGTKLEIK

SEQ ID NO: 24 - protein, 10 aa, synthetic construct
  SITE 1..10: note = anti BCMA antibody(J6M0) CDRH1
GGTFSNYWMH

SEQ ID NO: 25 - protein, 17 aa, synthetic construct
  SITE 1..17: note = anti BCMA antibody(J6M0) CDRH2
ATYRGHSDTYYNQKFKG

SEQ ID NO: 26 - protein, 12 aa, synthetic construct
  SITE 1..12: note = anti BCMA antibody(J6M0) CDRH3
GAIYDGYDVLDN

SEQ ID NO: 27 - protein, 11 aa, synthetic construct
  SITE 1..11: note = anti BCMA antibody(J6M0) CDRL1
SASQDISNYLN

SEQ ID NO: 28 - protein, 7 aa, synthetic construct
  SITE 1..7: note = anti BCMA antibody(J6M0) CDRL2
YTSNLHS

SEQ ID NO: 29 - protein, 9 aa, synthetic construct
  SITE 1..9: note = anti BCMA antibody(J6M0) CDRL3
QQYRKLPWT

SEQ ID NO: 30 - protein, 244 aa, synthetic construct
  SITE 1..244: note = J6M0 scfv
QVQLVQSGAEVKKPGSSVKVSCKASGGTFSNYWMHWVRQAPGQGLEWMGATYRGHSDTYYNQKFKGRVTITADKSTSTAYMELSSLRSEDTAVYYCARGAIYDGYDVLDNWGQGTLVTVSSGGGGSGGGGSGGGGSDIQMTQSPSSLSASVGDRVTITCSASQDISNYLNWYQQKPGKAPKLLIYYTSNLHSGVPSRFSGSGSGTDFTLTISSLQPEDFATYYCQQYRKLPWTFGQGTKLEIKR

SEQ ID NO: 31 - protein, 10 aa, synthetic construct
  SITE 1..10: note = anti BCMA antibody(BB2121) CDRH1
GYTFTDYSIN

SEQ ID NO: 32 - protein, 17 aa, synthetic construct
  SITE 1..17: note = anti BCMA antibody(BB2121) CDRH2
WINTETREPAYAYDFRG

SEQ ID NO: 33 - protein, 8 aa, synthetic construct
  SITE 1..8: note = anti BCMA antibody(BB2121) CDRH3
DYSYAMDY

SEQ ID NO: 34 - protein, 15 aa, synthetic construct
  SITE 1..15: note = anti BCMA antibody(BB2121) CDRL1
RASESVTILGSHLIH

SEQ ID NO: 35 - protein, 7 aa, synthetic construct
  SITE 1..7: note = anti BCMA antibody(BB2121) CDRL2
LASNVQT

SEQ ID NO: 36 - protein, 8 aa, synthetic construct
  SITE 1..8: note = anti BCMA antibody(BB2121) CDRL3
QSRTIPRT

SEQ ID NO: 37 - protein, 246 aa, synthetic construct
  SITE 1..246: note = BB2121 scfv
DIVLTQSPPSLAMSLGKRATISCRASESVTILGSHLIHWYQQKPGQPPTLLIQLASNVQTGVPARFSGSGSRTDFTLTIDPVEEDDVAVYYCLQSRTIPRTFGGGTKLEIKGSTSGSGKPGSGEGSTKGQIQLVQSGPELKKPGETVKISCKASGYTFTDYSINWVKRAPGKGLKWMGWINTETREPAYAYDFRGRFAFSLETSASTAYLQINNLKYEDTATYFCALDYSYAMDYWGQGTSVTVSS

SEQ ID NO: 38 - protein, 8 aa, synthetic construct
  SITE 1..8: note = anti CD22 antibody(m971) CDRH1
SSNSAAWN

SEQ ID NO: 39 - protein, 18 aa, synthetic construct
  SITE 1..18: note = anti CD22 antibody(m971) CDRH2
RTYYRSKWYNDYAVSVKS

SEQ ID NO: 40 - protein, 12 aa, synthetic construct
  SITE 1..12: note = anti CD22 antibody(m971) CDRH3
EVTGDLEDAFDI

SEQ ID NO: 41 - protein, 10 aa, synthetic construct
  SITE 1..10: note = anti CD22 antibody(m971) CDRL1
RASQTIWSYL

SEQ ID NO: 42 - protein, 7 aa, synthetic construct
  SITE 1..7: note = anti CD22 antibody(m971) CDRL2
AASSLQS

SEQ ID NO: 43 - protein, 9 aa, synthetic construct
  SITE 1..9: note = anti CD22 antibody(m971) CDRL3
QQSYSIPQT

SEQ ID NO: 44 - protein, 246 aa, synthetic construct
  SITE 1..246: note = m971 scfv
QVQLQQSGPGLVKPSQTLSLTCAISGDSVSSNSAAWNWIRQSPSRGLEWLGRTYYRSKWYNDYAVSVKSRITINPDTSKNQFSLQLNSVTPEDTAVYYCAREVTGDLEDAFDIWGQGTMVTVSSGGGGSGGGGSGGGGSDIQMTQSPSSLSASVGDRVTITCRASQTIWSYLNWYQQRPGKAPNLLIYAASSLQSGVPSRFSGRGSGTDFTLTISSLQAEDFATYYCQQSYSIPQTFGQGTKLEIK

SEQ ID NO: 45 - protein, 10 aa, synthetic construct
  SITE 1..10: note = anti CD22 antibody(LL2) CDRH1
GYTFTSYWLH

SEQ ID NO: 46 - protein, 17 aa, synthetic construct
  SITE 1..17: note = anti CD22 antibody(LL2) CDRH2
YINPRNDYTEYNQNFKD

SEQ ID NO: 47 - protein, 7 aa, synthetic construct
  SITE 1..7: note = anti CD22 antibody(LL2) CDRH3
RDITIFY

SEQ ID NO: 48 - protein, 16 aa, synthetic construct
  SITE 1..16: note = anti CD22 antibody(LL2) CDRL1
KSSQSVLYSANHKNYL

SEQ ID NO: 49 - protein, 7 aa, synthetic construct
  SITE 1..7: note = anti CD22 antibody(LL2) CDRL2
WASTRES

SEQ ID NO: 50 - protein, 8 aa, synthetic construct
  SITE 1..8: note = anti CD22 antibody(LL2) CDRL3
HQTLSSWT

SEQ ID NO: 51 - protein, 244 aa, synthetic construct
  SITE 1..244: note = LL2 scfv
QVQLVQSGAEVKKPGSSVKVSCKASGYTFTSYWLHWVRQAPGQGLEWIGYINPRNDYTEYNQNFKDKATITADESTNTAYMELSSLRSEDTAFYFCARRDITTFYWGQGTTVTVSSGGGGSGGGGSGGGGSDIQLTQSPSSLSASVGDRVTMSCKSSQSVLYSANHKNYLAWYQQKPGKAPKLLIYWASTRESGVPSRFSGSGSGTDFTFTISSLQPEDIATYYCHQYLSSWTFGGGTKLEIKR

SEQ ID NO: 52 - protein, 10 aa, synthetic construct
  SITE 1..10: note = anti CD22 antibody(G5/44) CDRH1
GYRFTNYWIH

SEQ ID NO: 53 - protein, 17 aa, synthetic construct
  SITE 1..17: note = anti CD22 antibody(G5/44) CDRH2
GINPGNNYATYRRKFQG

SEQ ID NO: 54 - protein, 12 aa, synthetic construct
  SITE 1..12: note = anti CD22 antibody(G5/44) CDRH3
EGYGNYGAWFAY

SEQ ID NO: 55 - protein, 15 aa, synthetic construct
  SITE 1..15: note = anti CD22 antibody(G5/44) CDRL1
RSSQSLANSYGNTFL

SEQ ID NO: 56 - protein, 7 aa, synthetic construct
  SITE 1..7: note = anti CD22 antibody(G5/44) CDRL2
GISNRFS

SEQ ID NO: 57 - protein, 9 aa, synthetic construct
  SITE 1..9: note = anti CD22 antibody(G5/44) CDRL3
LQGTHQPYT

SEQ ID NO: 58 - protein, 249 aa, synthetic construct
  SITE 1..249: note = G5/44 scfv
EVQLVQSGAEVKKPGASVKVSCKASGYRFTNYWIHWVRQAPGQGLEWIGGINPGNNYATYRRKFQGRVTMTADTSTSTVYMELSSLRSEDTAVYYCTREGYGNYGAWFAYWGQGTLVTVSSGGGGSGGGGSGGGGSDVQVTQSPSSLSASVGDRVTITCRSSQSLANSYGNTFLSWYLHKPGKAPQLLIYGISNRFSGVPDRFSGSGSGTDFTLTISSLQPEDFATYYCLQGTHQPYTFGQGTKVEIKR

SEQ ID NO: 59 - protein, 10 aa, synthetic construct
  SITE 1..10: note = anti CD22 antibody(RFB4) CDRH1
GFTFSIYDMS

SEQ ID NO: 60 - protein, 17 aa, synthetic construct
  SITE 1..17: note = anti CD22 antibody(RFB4) CDRH2
YISSGGGTTYYPDTVKG

SEQ ID NO: 61 - protein, 14 aa, synthetic construct
  SITE 1..14: note = anti CD22 antibody(RFB4) CDRH3
HSGYGSSYGVLFAY

SEQ ID NO: 62 - protein, 10 aa, synthetic construct
  SITE 1..10: note = anti CD22 antibody(RFB4) CDRL1
RASQTISNYL

SEQ ID NO: 63 - protein, 7 aa, synthetic construct
  SITE 1..7: note = anti CD22 antibody(RFB4) CDRL2
YTSILHS

SEQ ID NO: 64 - protein, 9 aa, synthetic construct
  SITE 1..9: note = anti CD22 antibody(RFB4) CDRL3
QQGNTLPWT

SEQ ID NO: 65 - protein, 244 aa, synthetic construct
  SITE 1..244: note = RFB4 scfv
QLVQSGAEVKKPGSSVKVSCKASGFTFSIYDMSWVRQAPGQGLEWVAYISSGGGTTYYPDTVKGRFTITADESTNTAYMELSSLRSEDTAFYFCARHSGYGSSYGVLFAYWGQGTLVTVSSGGGGSGGGGSGGGGSDIQLTQSPSSLSASVGDRVTISCRASQDISNYLNWYQQKPGKAPKLLIYYTSILHSGVPSRFSGSGSGTDYTFTISSLQPEDIATYYCQQGNTLPWTFGGGTKVQIKR

SEQ ID NO: 66 - DNA, 45 bp, synthetic construct
  source 1..45: mol_type = other DNA
  misc_feature 1..45: note = (G4S)3 hinge
ggcggcggaggctctggcggcggcggcagcggcggcggaggctcc

SEQ ID NO: 67 - DNA, 207 bp, synthetic construct
  source 1..207: mol_type = other DNA
  misc_feature 1..207: note = CD8 hinge
accactaccccagcaccgaggccacccaccccggctcctaccatcgcctcccagcctctgtccctgcgtccggaggcatgtagacccgcagctggtggggccgtgcatacccggggtcttgacttcgcctgcgatatctacatttgggcccctctggctggtacttgcggggtcctgctgctttcactcgtgatcactctttactgt

SEQ ID NO: 68 - DNA, 117 bp, synthetic construct
  source 1..117: mol_type = other DNA
  misc_feature 1..117: note = CD28 hinge
attgaagttatgtatcctcctccttacctagacaatgagaagagcaatggaaccattatccatgtgaaagggaaacacctttgtccaagtcccctatttcccggaccttctaagccc

SEQ ID NO: 69 - DNA, 36 bp, synthetic construct
  source 1..36: mol_type = other DNA
  misc_feature 1..36: note = IgG4 hinge
gagtccaaatatggtcccccatgcccatcatgccca

SEQ ID NO: 70 - DNA, 30 bp, synthetic construct
  source 1..30: mol_type = other DNA
  misc_feature 1..30: note = EAAAKGGGGS hinge
gaagcggcggcgaaaggaggaggaggaagc

SEQ ID NO: 71 - DNA, 45 bp, synthetic construct
  source 1..45: mol_type = other DNA
  misc_feature 1..45: note = (EAAAK)3 hinge
gaagcagccgctaaagaggcagctgctaaggaagccgcagctaaa

SEQ ID NO: 72 - DNA, 54 bp, synthetic construct
  source 1..54: mol_type = other DNA
  misc_feature 1..54: note = GST hinge
ggaagcacgtccggctcagggaagccgggctccggcgagggaagcacgaagggg

SEQ ID NO: 73 - DNA, 60 bp, synthetic construct
  source 1..60: mol_type = other DNA
  misc_feature 1..60: note = EAAAK-GS hinge
gaagcagccgctaaaggcggaggcggttctggaggcggtggctccgcggccgcagctaag

SEQ ID NO: 74 - DNA, 192 bp, synthetic construct
  source 1..192: mol_type = other DNA
  misc_feature 1..192: note = IgD hinge
aggtggcccgaaagtcccaaggcccaggcatctagtgttcctactgcacagccccaggcagaaggcagcctagccaaagctactactgcacctgccactacgcgcaatactggccgtggcggggaggagaagaaaaaggagaaagagaaagaagaacaggaagagagggagaccaagacccctgaatgtcca

SEQ ID NO: 75 - DNA, 357 bp, synthetic construct
  source 1..357: mol_type = other DNA
  misc_feature 1..357: note = IgG4-CH3 hinge
gagtccaaatatggtcccccatgcccatcatgcccagggcagccccgagagccacaggtgtacaccctgcccccatcccaggaggagatgaccaagaaccaggtcagcctgacctgcctggtcaaaggcttctaccccagcgacatcgccgtggagtgggagagcaatgggcagccggagaacaactacaagaccacgcctcccgtgctggactccgacggctccttcttcctctacagcaggctaaccgtggacaagagcaggtggcaggaggggaatgtcttctcatgctccgtgatgcatgaggctctgcacaaccactacacacagaagagcctctccctgtctctgggtaaa

SEQ ID NO: 76 - DNA, 36 bp, synthetic construct
  source 1..36: mol_type = other DNA
  misc_feature 1..36: note = (AP)6 hinge
gcacctgcccctgcaccagctccagctcccgcccca

SEQ ID NO: 77 - DNA, 258 bp, synthetic construct
  source 1..258: mol_type = other DNA
  misc_feature 1..258: note = DNA sequence of Fc epsilon R1 gamma
atgattccagcagtggtcttgctcttactccttttggttgaacaagcagcggccctgggagagcctcagctctgctatatcctggatgccatcctgtttctgtatggaattgtcctcaccctcctctactgtcgactgaagatccaagtgcgaaaggcagctataaccagctatgagaaatcagatggtgtttacacgggcctgagcaccaggaaccaggagacttacgagactctgaagcatgagaaaccaccacag

SEQ ID NO: 78 - DNA, 726 bp, synthetic construct
  source 1..726: mol_type = other DNA
  misc_feature 1..726: note = FMC63 scfv (DNA sequence)
gacatccagatgacacagactacatcctccctgtctgcctctctgggagacagagtcaccatcagttgcagggcaagtcaggacattagtaaatatttaaattggtatcagcagaaaccagatggaactgttaaactcctgatctaccatacatcaagattacactcaggagtcccatcaaggttcagtggcagtgggtctggaacagattattctctcaccattagcaacctggagcaagaagatattgccacttacttttgccaacagggtaatacgcttccgtacacgttcggaggggggaccaagctggagatcacaggtggcggtggctcgggcggtggtgggtcgggtggcggcggatctgaggtgaaactgcaggagtcaggacctggcctggtggcgccctcacagagcctgtccgtcacatgcactgtctcaggggtctcattacccgactatggtgtaagctggattcgccagcctccacgaaagggtctggagtggctgggagtaatatggggtagtgaaaccacatactataattcagctctcaaatccagactgaccatcatcaaggacaactccaagagccaagttttcttaaaaatgaacagtctgcaaactgatgacacagccatttactactgtgccaaacattattactacggtggtagctatgctatggactactggggccaaggaacctcagtcaccgtctcctca

SEQ ID NO: 79 - DNA, 225 bp, synthetic construct
  source 1..225: mol_type = other DNA
  misc_feature 1..225: note = NKp30 without Ig-like domain (DNA sequence)
gtggagaaggagcaccctcagctgggagcaggcaccgtgctgctgctgagggccggcttctatgccgtgagctttctgtccgtggccgtgggctccaccgtgtactatcagggcaagtgcctgacatggaaaggcccccggagacagctgccagccgtggtgccagcaccactgcctccaccctgtggctcctctgcccacctgctgcctccagtgcccggcggc

SEQ ID NO: 80 - DNA, 63 bp, synthetic construct
  source 1..63: mol_type = other DNA
  misc_feature 1..63: note = T2A (DNA sequence)
ggctctggagagggaagaggcagcctgctgacctgcggcgacgtggaggagaatcctggccca

SEQ ID NO: 81 - DNA, 1407 bp, synthetic construct
  source 1..1407: mol_type = other DNA
  misc_feature 1..1407: note = the nucleic acid molecule of example 1-1
atgatcccagccgtggtgctgctgctgctgctgctggtggagcaggccgccgccctgggagagccccagctgtgctacatcctggacgccatcctgttcctgtacggcatcgtgctgaccctgctgtattgtaggctgaagatccaggtgcgcaaggccgccatcacatcttacgagaagagcgatggcgtgtataccggcctgagcacaagaaaccaggagacatacgagacactgaagcacgagaagccacctcagggctctggagagggaagaggcagcctgctgacctgcggcgacgtggaggagaatcctggcccaatcgatgccaccatggccttaccagtgaccgccttgctcctgccgctggccttgctgctccacgccgccaggccggacatccagatgacacagactacatcctccctgtctgcctctctgggagacagagtcaccatcagttgcagggcaagtcaggacattagtaaatatttaaattggtatcagcagaaaccagatggaactgttaaactcctgatctaccatacatcaagattacactcaggagtcccatcaaggttcagtggcagtgggtctggaacagattattctctcaccattagcaacctggagcaagaagatattgccacttacttttgccaacagggtaatacgcttccgtacacgttcggaggggggaccaagctggagatcacaggtggcggtggctcgggcggtggtgggtcgggtggcggcggatctgaggtgaaactgcaggagtcaggacctggcctggtggcgccctcacagagcctgtccgtcacatgcactgtctcaggggtctcattacccgactatggtgtaagctggattcgccagcctccacgaaagggtctggagtggctgggagtaatatggggtagtgaaaccacatactataattcagctctcaaatccagactgaccatcatcaaggacaactccaagagccaagttttcttaaaaatgaacagtctgcaaactgatgacacagccatttactactgtgccaaacattattactacggtggtagctatgctatggactactggggccaaggaacctcagtcaccgtctcctcaactagtggcggcggaggctctggcggcggcggcagcggcggcggaggctccgctagcgtggagaaggagcaccctcagctgggagcaggcaccgtgctgctgctgagggccggcttctatgccgtgagctttctgtccgtggccgtgggctccaccgtgtactatcagggcaagtgcctgacatggaaaggcccccggagacagctgccagccgtggtgccagcaccactgcctccaccctgtggctcctctgcccacctgctgcctccagtgcccggcggctga

SEQ ID NO: 82 - DNA, 1476 bp, synthetic construct
  source 1..1476: mol_type = other DNA
  misc_feature 1..1476: note = the nucleic acid molecule of example 1-2
atgattccagcagtggtcttgctcttactccttttggttgaacaagcagcggccctgggagagcctcagctctgctatatcctggatgccatcctgtttctgtatggaattgtcctcaccctcctctactgtcgactgaagatccaagtgcgaaaggcagctataaccagctatgagaaatcagatggtgtttacacgggcctgagcaccaggaaccaggagacttacgagactctgaagcatgagaaaccaccacagggctctggagagggaagaggcagcctgctgacctgcggcgacgtggaggagaatcctggcccaatcgatgccaccatcgatgccaccatggccttaccagtgaccgccttgctcctgccgctggccttgctgctccacgccgccaggccggacatccagatgacacagactacatcctccctgtctgcctctctgggagacagagtcaccatcagttgcagggcaagtcaggacattagtaaatatttaaattggtatcagcagaaaccagatggaactgttaaactcctgatctaccatacatcaagattacactcaggagtcccatcaaggttcagtggcagtgggtctggaacagattattctctcaccattagcaacctggagcaagaagatattgccacttacttttgccaacagggtaatacgcttccgtacacgttcggaggggggaccaagctggagatcacaggtggcggtggctcgggcggtggtgggtcgggtggcggcggatctgaggtgaaactgcaggagtcaggacctggcctggtggcgccctcacagagcctgtccgtcacatgcactgtctcaggggtctcattacccgactatggtgtaagctggattcgccagcctccacgaaagggtctggagtggctgggagtaatatggggtagtgaaaccacatactataattcagctctcaaatccagactgaccatcatcaaggacaactccaagagccaagttttcttaaaaatgaacagtctgcaaactgatgacacagccatttactactgtgccaaacattattactacggtggtagctatgctatggactactggggccaaggaacctcagtcaccgtctcctcaattgaagttatgtatcctcctccttacctagacaatgagaagagcaatggaaccattatccatgtgaaagggaaacacctttgtccaagtcccctatttcccggaccttctaagcccgtggagaaggagcaccctcagctgggagcaggcaccgtgctgctgctgagggccggcttctatgccgtgagctttctgtccgtggccgtgggctccaccgtgtactatcagggcaagtgcctgacatggaaaggcccccggagacagctgccagccgtggtgccagcaccactgcctccaccctgtggctcctctgcccacctgctgcctccagtgcccggcggc

SEQ ID NO: 83 - DNA, 1488 bp, synthetic construct
  source 1..1488: mol_type = other DNA
  misc_feature 1..1488: note = the nucleic acid molecule of example 1-3
atgatcccagccgtggtgctgctgctgctgctgctggtggagcaggccgccgccctgggagagccccagctgtgctacatcctggacgccatcctgttcctgtacggcatcgtgctgaccctgctgtattgtaggctgaagatccaggtgcgcaaggccgccatcacatcttacgagaagagcgatggcgtgtataccggcctgagcacaagaaaccaggagacatacgagacactgaagcacgagaagccacctcagggctctggagagggaagaggcagcctgctgacctgcggcgacgtggaggagaatcctggcccaatcgatgccaccatggccttaccagtgaccgccttgctcctgccgctggccttgctgctccacgccgccaggccggacatccagatgacacagactacatcctccctgtctgcctctctgggagacagagtcaccatcagttgcagggcaagtcaggacattagtaaatatttaaattggtatcagcagaaaccagatggaactgttaaactcctgatctaccatacatcaagattacactcaggagtcccatcaaggttcagtggcagtgggtctggaacagattattctctcaccattagcaacctggagcaagaagatattgccacttacttttgccaacagggtaatacgcttccgtacacgttcggaggggggaccaagctggagatcacaggtggcggtggctcgggcggtggtgggtcgggtggcggcggatctgaggtgaaactgcaggagtcaggacctggcctggtggcgccctcacagagcctgtccgtcacatgcactgtctcaggggtctcattacccgactatggtgtaagctggattcgccagcctccacgaaagggtctggagtggctgggagtaatatggggtagtgaaaccacatactataattcagctctcaaatccagactgaccatcatcaaggacaactccaagagccaagttttcttaaaaatgaacagtctgcaaactgatgacacagccatttactactgtgccaaacattattactacggtggtagctatgctatggactactggggccaaggaacctcagtcaccgtctcctcaaccactaccccagcaccgaggccacccaccccggctcctaccatcgcctcccagcctctgtccctgcgtccggaggcatgtagacccgcagctggtggggccgtgcatacccggggtcttgacttcgcctgcgatatctacgtggagaaggagcaccctcagctgggagcaggcaccgtgctgctgctgagggccggcttctatgccgtgagctttctgtccgtggccgtgggctccaccgtgtactatcagggcaagtgcctgacatggaaaggcccccggagacagctgccagccgtggtgccagcaccactgcctccaccctgtggctcctctgcccacctgctgcctccagtgcccggcggc

SEQ ID NO: 84 - DNA, 1383 bp, synthetic construct
  source 1..1383: mol_type = other DNA
  misc_feature 1..1383: note = the nucleic acid molecule of example 1-4
atgatcccagccgtggtgctgctgctgctgctgctggtggagcaggccgccgccctgggagagccccagctgtgctacatcctggacgccatcctgttcctgtacggcatcgtgctgaccctgctgtattgtaggctgaagatccaggtgcgcaaggccgccatcacatcttacgagaagagcgatggcgtgtataccggcctgagcacaagaaaccaggagacatacgagacactgaagcacgagaagccacctcagggctctggagagggaagaggcagcctgctgacctgcggcgacgtggaggagaatcctggcccaatcgatgccaccatggccttaccagtgaccgccttgctcctgccgctggccttgctgctccacgccgccaggccggacatccagatgacacagactacatcctccctgtctgcctctctgggagacagagtcaccatcagttgcagggcaagtcaggacattagtaaatatttaaattggtatcagcagaaaccagatggaactgttaaactcctgatctaccatacatcaagattacactcaggagtcccatcaaggttcagtggcagtgggtctggaacagattattctctcaccattagcaacctggagcaagaagatattgccacttacttttgccaacagggtaatacgcttccgtacacgttcggaggggggaccaagctggagatcacaggtggcggtggctcgggcggtggtgggtcgggtggcggcggatctgaggtgaaactgcaggagtcaggacctggcctggtggcgccctcacagagcctgtccgtcacatgcactgtctcaggggtctcattacccgactatggtgtaagctggattcgccagcctccacgaaagggtctggagtggctgggagtaatatggggtagtgaaaccacatactataattcagctctcaaatccagactgaccatcatcaaggacaactccaagagccaagttttcttaaaaatgaacagtctgcaaactgatgacacagccatttactactgtgccaaacattattactacggtggtagctatgctatggactactggggccaaggaacctcagtcaccgtctcctcagagtccaaatatggtcccccatgcccatcatgcccagtggagaaggagcaccctcagctgggagcaggcaccgtgctgctgctgagggccggcttctatgccgtgagctttctgtccgtggccgtgggctccaccgtgtactatcagggcaagtgcctgacatggaaaggcccccggagacagctgccagccgtggtgccagcaccactgcctccaccctgtggctcctctgcccacctgctgcctccagtgcccggcggc

SEQ ID NO: 85 - DNA, 1404 bp, synthetic construct
  source 1..1404: mol_type = other DNA
  misc_feature 1..1404: note = the nucleic acid molecule of example 1-5
atgatcccagccgtggtgctgctgctgctgctgctggtggagcaggccgccgccctgggagagccccagctgtgctacatcctggacgccatcctgttcctgtacggcatcgtgctgaccctgctgtattgtaggctgaagatccaggtgcgcaaggccgccatcacatcttacgagaagagcgatggcgtgtataccggcctgagcacaagaaaccaggagacatacgagacactgaagcacgagaagccacctcagggctctggagagggaagaggcagcctgctgacctgcggcgacgtggaggagaatcctggcccaatcgatgccaccatggccttaccagtgaccgccttgctcctgccgctggccttgctgctccacgccgccaggccggacatccagatgacacagactacatcctccctgtctgcctctctgggagacagagtcaccatcagttgcagggcaagtcaggacattagtaaatatttaaattggtatcagcagaaaccagatggaactgttaaactcctgatctaccatacatcaagattacactcaggagtcccatcaaggttcagtggcagtgggtctggaacagattattctctcaccattagcaacctggagcaagaagatattgccacttacttttgccaacagggtaatacgcttccgtacacgttcggaggggggaccaagctggagatcacaggtggcggtggctcgggcggtggtgggtcgggtggcggcggatctgaggtgaaactgcaggagtcaggacctggcctggtggcgccctcacagagcctgtccgtcacatgcactgtctcaggggtctcattacccgactatggtgtaagctggattcgccagcctccacgaaagggtctggagtggctgggagtaatatggggtagtgaaaccacatactataattcagctctcaaatccagactgaccatcatcaaggacaactccaagagccaagttttcttaaaaatgaacagtctgcaaactgatgacacagccatttactactgtgccaaacattattactacggtggtagctatgctatggactactggggccaaggaacctcagtcaccgtctcctcaactagtgaagcagccgctaaagaggcagctgctaaggaagccgcagctaaagctagcgtggagaaggagcaccctcagctgggagcaggcaccgtgctgctgctgagggccggcttctatgccgtgagctttctgtccgtggccgtgggctccaccgtgtactatcagggcaagtgcctgacatggaaaggcccccggagacagctgccagccgtggtgccagcaccactgcctccaccctgtggctcctctgcccacctgctgcctccagtgcccggcggc

SEQ ID NO: 86 - DNA, 207 bp, synthetic construct; identical to SEQ ID NO: 67
  source 1..207: mol_type = other DNA
  misc_feature 1..207: note = CD8 transmembrane domain (DNA sequence)

SEQ ID NO: 87 - DNA, 126 bp, synthetic construct
  source 1..126: mol_type = other DNA
  misc_feature 1..126: note = 4-1BB signaling domain (DNA sequence)
aagcgcggtcggaagaagctgctgtacatctttaagcaacccttcatgaggcctgtgcagactactcaagaggaggacggctgttcatgccggttcccagaggaggaggaaggcggctgcgaactg

SEQ ID NO: 88 - DNA, 336 bp, synthetic construct
  source 1..336: mol_type = other DNA
  misc_feature 1..336: note = CD3 zeta signaling domain (DNA sequence)
cgcgtgaaattcagccgcagcgcagatgctccagcctacaagcaggggcagaaccagctctacaacgaactcaatcttggtcggagagaggagtacgacgtgctggacaagcggagaggacgggacccagaaatgggcgggaagccgcgcagaaagaatccccaagagggcctgtacaacgagctccaaaaggataagatggcagaagcctatagcgagattggtatgaaaggggaacgcagaagaggcaaaggccacgacggactgtaccagggactcagcaccgccaccaaggacacctatgacgctcttcacatgcaggccctgccgcctcgg

SEQ ID NO: 89 - DNA, 1395 bp, synthetic construct
  source 1..1395: mol_type = other DNA
  misc_feature 1..1395: note = the nucleic acid molecule of comparative example 1
gacatccagatgacacagactacatcctccctgtctgcctctctgggagacagagtcaccatcagttgcagggcaagtcaggacattagtaaatatttaaattggtatcagcagaaaccagatggaactgttaaactcctgatctaccatacatcaagattacactcaggagtcccatcaaggttcagtggcagtgggtctggaacagattattctctcaccattagcaacctggagcaagaagatattgccacttacttttgccaacagggtaatacgcttccgtacacgttcggaggggggaccaagctggagatcacaggtggcggtggctcgggcggtggtgggtcgggtggcggcggatctgaggtgaaactgcaggagtcaggacctggcctggtggcgccctcacagagcctgtccgtcacatgcactgtctcaggggtctcattacccgactatggtgtaagctggattcgccagcctccacgaaagggtctggagtggctgggagtaatatggggtagtgaaaccacatactataattcagctctcaaatccagactgaccatcatcaaggacaactccaagagccaagttttcttaaaaatgaacagtctgcaaactgatgacacagccatttactactgtgccaaacattattactacggtggtagctatgctatggactactggggccaaggaacctcagtcaccgtctcctcaaccactaccccagcaccgaggccacccaccccggctcctaccatcgcctcccagcctctgtccctgcgtccggaggcatgtagacccgcagctggtggggccgtgcatacccggggtcttgacttcgcctgcgatatctacatttgggcccctctggctggtacttgcggggtcctgctgctttcactcgtgatcactctttactgtaagcgcggtcggaagaagctgctgtacatctttaagcaacccttcatgaggcctgtgcagactactcaagaggaggacggctgttcatgccggttcccagaggaggaggaaggcggctgcgaactgcgcgtgaaattcagccgcagcgcagatgctccagcctacaagcaggggcagaaccagctctacaacgaactcaatcttggtcggagagaggagtacgacgtgctggacaagcggagaggacgggacccagaaatgggcgggaagccgcgcagaaagaatccccaagagggcctgtacaacgagctccaaaaggataagatggcagaagcctatagcgagattggtatgaaaggggaacgcagaagaggcaaaggccacgacggactgtaccagggactcagcaccgccaccaaggacacctatgacgctcttcacatgcaggccctgccgcctcgg

SEQ ID NO: 90 - DNA, 1026 bp, Homo sapiens
  source 1..1026: mol_type = genomic DNA
  misc_feature 1..1026: note = truncated CD19 fragment (DNA sequence)
atgccacctcctcgcctcctcttcttcctcctcttcctcacccccatggaagtcaggcccgaggaacctctagtggtgaaggtggaagagggagataacgctgtgctgcagtgcctcaaggggacctcagatggccccactcagcagctgacctggtctcgggagtccccgcttaaacccttcttaaaactcagcctggggctgccaggcctgggaatccacatgaggcccctggccatctggcttttcatcttcaacgtctctcaacagatggggggcttctacctgtgccagccggggcccccctctgagaaggcctggcagcctggctggacagtcaatgtggagggcagcggggagctgttccggtggaatgtttcggacctaggtggcctgggctgtggcctgaagaacaggtcctcagagggccccagctccccttccgggaagctcatgagccccaagctgtatgtgtgggccaaagaccgccctgagatctgggagggagagcctccgtgtctcccaccgagggacagcctgaaccagagcctcagccaggacctcaccatggcccctggctccacactctggctgtcctgtggggtaccccctgactctgtgtccaggggccccctctcctggacccatgtgcaccccaaggggcctaagtcattgctgagcctagagctgaaggacgatcgcccggccagagatatgtgggtaatggagacgggtctgttgttgccccgggccacagctcaagacgctggaaagtattattgtcaccgtggcaacctgaccatgtcattccacctggagatcactgctcggccagtactatggcactggctgctgaggactggtggctggaaggtctcagctgtgactttggcttatctgatcttctgcctgtgttcccttgtgggcattcttcatcttcaaagagccctggtcctgaggaggaaaagaaagcgaatgactgaccccaccaggagattcttcaaagtgacgcctcccccaggaagc

SEQ ID NO: 91 - DNA, 720 bp, synthetic construct
  source 1..720: mol_type = other DNA
  misc_feature 1..720: note = SS1 scfv (DNA sequence)
caggtgcagctccagcagtccggcccagagctggagaagcctggcgcctctgtgaagctgagctgtaaggccagcggctactccttcaccggctatacaatgaactgggtgaagcagtcccacggcaagtctctggagtggatcggcctgatcaccccctacaacggcgccagctcctataatcagaagtttcgcggcaaggccaccctgacagtggataagtctagctccaccgcctacatggacctgctgtctctgacaagcgaggattccgccgtgtacttctgcgccagaggcggctatgacggcagaggctttgattactggggccagggcaccacagtgaccgtgtctagcggcgtgggcggctctggaggaggaggcagcggcggaggaggctccgacatcgagctgacacagtccccagcaatcatgtctgccagccccggcgagaaggtgaccatgacatgttccgcctcctctagcgtgtcttacatgcactggtatcagcagaagtctggcaccagccctaagaggtggatctatgatacaagcaagctggcatccggcgtgccaggccgcttctccggctctggcagcggcaattcctactctctgaccatctcctctgtggaggccgaggacgatgccacatactattgccagcagtggagcaagcacccactgacctttggcgccggcacaaagctggagatcaag

SEQ ID NO: 92 - DNA, 1386 bp, synthetic construct
  source 1..1386: mol_type = other DNA
  misc_feature 1..1386: note = the nucleic acid molecule of example 2
atgatccccgccgtggtgctgctgctgctgctgctggtggagcaggccgccgccctgggagagcctcagctgtgctatatcctggacgccatcctgttcctgtatggcatcgtgctgaccctgctgtactgtaggctgaagatccaggtgcgcaaggccgccatcacaagctacgagaagtccgatggcgtgtataccggcctgagcacacggaaccaggagacatacgagacactgaagcacgagaagccacctcagggctctggagagggaagaggcagcctgctgacctgcggcgacgtggaggagaatcctggcccagcaagcatggccctgccagtgacagccctgctgctgcctctggccctgctgctgcacgcagccaggcctcaggtgcagctccagcagtccggcccagagctggagaagcctggcgcctctgtgaagctgagctgtaaggccagcggctactccttcaccggctatacaatgaactgggtgaagcagtcccacggcaagtctctggagtggatcggcctgatcaccccctacaacggcgccagctcctataatcagaagtttcgcggcaaggccaccctgacagtggataagtctagctccaccgcctacatggacctgctgtctctgacaagcgaggattccgccgtgtacttctgcgccagaggcggctatgacggcagaggctttgattactggggccagggcaccacagtgaccgtgtctagcggcgtgggcggctctggaggaggaggcagcggcggaggaggctccgacatcgagctgacacagtccccagcaatcatgtctgccagccccggcgagaaggtgaccatgacatgttccgcctcctctagcgtgtcttacatgcactggtatcagcagaagtctggcaccagccctaagaggtggatctatgatacaagcaagctggcatccggcgtgccaggccgcttctccggctctggcagcggcaattcctactctctgaccatctcctctgtggaggccgaggacgatgccacatactattgccagcagtggagcaagcacccactgacctttggcgccggcacaaagctggagatcaagattgacggcggcggaggctctggcggcggcggcagcggcggcggaggctccgtggagaaggagcacccccagctgggagcaggcaccgtgctgctgctgagggcaggcttctacgccgtgtcctttctgtctgtggccgtgggctccaccgtgtactatcagggcaagtgcctgacatggaaaggcccccggagacagctgccagccgtggtgcccgcacctctgccaccaccttgtggcagctccgcccacctgctgccacccgtgcccggcggc

SEQ ID NO: 93 - DNA, 1395 bp, synthetic construct
  source 1..1395: mol_type = other DNA
  misc_feature 1..1395: note = the nucleic acid molecule of comparative example 2
caggtacaactgcagcagtctgggcctgagctggagaagcctggcgcttcagtgaagctgtcctgcaaggcttctggttactcattcactggctacaccatgaactgggtgaagcagagccatggaaagagccttgagtggattggacttattactccttacaatggtgcttctagctacaaccagaagttcaggggcaaggccacattaactgtagacaagtcatccagcacagcctacatggacctcctcagtctgacatctgaagactctgcagtctatttctgtgcaagggggggttacgacgggaggggttttgactactggggccaagggaccacggtcaccgtctcctcaggtgtaggcggttcaggcggcggtggctctggcggtggcggatcggacatcgagctcactcagtctccagcaatcatgtctgcatctccaggggagaaggtcaccatgacctgcagtgccagctcaagtgtaagttacatgcactggtatcagcagaagtcaggcacctcccccaaaagatggatttatgacacatccaaactggcttctggagtcccaggtcgcttcagtggcagtgggtctggaaactcttactctctcacaatcagcagcgtggaggctgaagatgatgcaacttattactgccagcagtggagtaagcatcctctcacgttcggtgctgggacaaagttggaaataaaaaccactaccccagcaccgaggccacccaccccggctcctaccatcgcctcccagcctctgtccctgcgtccggaggcatgtagacccgcagctggtggggccgtgcatacccgaggtcttgacttcgcctgcgacatctacatttgggcccctctggctggtacttgcggggtcctgctgctttcactcgtgatcactctttactgtaagcgcggtcggaagaagctgctgtacatctttaagcaacccttcatgaggcctgtgcagactactcaagaggaggacggctgttcatgccggttcccagaggaggaggaaggcggctgcgaactgcgcgtgaaattcagccgcagcgcagatgctccagcctacaagcaggggcagaaccagctctacaacgaactcaatcttggtcggagagaggagtacgacgtgctggacaagcggagaggacgggacccagaaatgggcgggaagccgcgcagaaagaatccccaagagggcctgtacaacgagctccaaaaggataagatggcagaagcctatagcgagattggtatgaaaggggaacgcagaagaggcaaaggccacgacggactgtaccagggactcagcaccgccaccaaggacacctatgacgctcttcacatgcaggccctgccgcctcgggctagc

SEQ ID NO: 94 - DNA, 732 bp, synthetic construct
  source 1..732: mol_type = other DNA
  misc_feature 1..732: note = J6M0 scfv (DNA sequence)
caggtccagctggtccagtccggagccgaggtgaagaagcctggcagctccgtgaaggtgagctgcaaggcctccggcggcacattcagcaactactggatgcactgggtgcgccaggcaccaggacagggcctggagtggatgggcgccacatatcgcggccactccgatacctactataatcagaagtttaagggccgggtgacaatcaccgccgacaagtccacatctaccgcctacatggagctgtctagcctgagatccgaggataccgccgtgtactattgcgccaggggcgccatctacgacggctatgatgtgctggacaactggggccagggcacactggtgaccgtgtcctctggaggaggaggctccggcggaggaggctctggcggcggcggcagcgacatccagatgacacagtcccccagctccctgagcgcctccgtgggcgatagagtgacaatcacctgttctgccagccaggacatctctaactacctgaattggtatcagcagaagcccggcaaggcccctaagctgctgatctactatacctctaatctgcacagcggcgtgccttcccgcttctccggctctggcagcggcacagacttcaccctgaccatctctagcctgcagcccgaggacttcgccacctactattgccagcagtaccggaagctgccttggacatttggccagggcaccaagctggagatcaagagg

SEQ ID NO: 95 - DNA, 1467 bp, synthetic construct
  source 1..1467: mol_type = other DNA
  misc_feature 1..1467: note = the nucleic acid molecule of example 3
atgatcccagccgtggtgctgctgctgctgctgctggtggagcaggccgccgccctgggagagccccagctgtgctacatcctggacgccatcctgttcctgtacggcatcgtgctgaccctgctgtattgtaggctgaagatccaggtgcgcaaggccgccatcacatcttacgagaagagcgatggcgtgtataccggcctgagcacaagaaaccaggagacatacgagacactgaagcacgagaagccacctcagggctctggagagggaagaggcagcctgctgacctgcggcgacgtggaggagaatcctggcccaatcgatgccaccatggccttaccagtgaccgccttgctcctgccgctggccttgctgctccacgccgccaggccgcaggtccagctggtccagtccggagccgaggtgaagaagcctggcagctccgtgaaggtgagctgcaaggcctccggcggcacattcagcaactactggatgcactgggtgcgccaggcaccaggacagggcctggagtggatgggcgccacatatcgcggccactccgatacctactataatcagaagtttaagggccgggtgacaatcaccgccgacaagtccacatctaccgcctacatggagctgtctagcctgagatccgaggataccgccgtgtactattgcgccaggggcgccatctacgacggctatgatgtgctggacaactggggccagggcacactggtgaccgtgtcctctggaggaggaggctccggcggaggaggctctggcggcggcggcagcgacatccagatgacacagtcccccagctccctgagcgcctccgtgggcgatagagtgacaatcacctgttctgccagccaggacatctctaactacctgaattggtatcagcagaagcccggcaaggcccctaagctgctgatctactatacctctaatctgcacagcggcgtgccttcccgcttctccggctctggcagcggcacagacttcaccctgaccatctctagcctgcagcccgaggacttcgccacctactattgccagcagtaccggaagctgccttggacatttggccagggcaccaagctggagatcaagattgaagttatgtatcctcctccttacctagacaatgagaagagcaatggaaccattatccatgtgaaagggaaacacctttgtccaagtcccctatttcccggaccttctaagcccgtggagaaggagcaccctcagctgggagcaggcaccgtgctgctgctgagggccggcttctatgccgtgagctttctgtccgtggccgtgggctccaccgtgtactatcagggcaagtgcctgacatggaaaggcccccggagacagctgccagccgtggtgccagcaccactgcctccaccctgtggctcctctgcccacctgctgcctccagtgcccggcggc

SEQ ID NO: 96 - DNA, 1401 bp, synthetic construct
  source 1..1401: mol_type = other DNA
  misc_feature 1..1401: note = the nucleic acid molecule of comparative example 3
caggtccagctggtccagtccggagccgaggtgaagaagcctggcagctccgtgaaggtgagctgcaaggcctccggcggcacattcagcaactactggatgcactgggtgcgccaggcaccaggacagggcctggagtggatgggcgccacatatcgcggccactccgatacctactataatcagaagtttaagggccgggtgacaatcaccgccgacaagtccacatctaccgcctacatggagctgtctagcctgagatccgaggataccgccgtgtactattgcgccaggggcgccatctacgacggctatgatgtgctggacaactggggccagggcacactggtgaccgtgtcctctggaggaggaggctccggcggaggaggctctggcggcggcggcagcgacatccagatgacacagtcccccagctccctgagcgcctccgtgggcgatagagtgacaatcacctgttctgccagccaggacatctctaactacctgaattggtatcagcagaagcccggcaaggcccctaagctgctgatctactatacctctaatctgcacagcggcgtgccttcccgcttctccggctctggcagcggcacagacttcaccctgaccatctctagcctgcagcccgaggacttcgccacctactattgccagcagtaccggaagctgccttggacatttggccagggcaccaagctggagatcaagaggaccacaaccccagcaccccggccccctacacctgccccaaccatcgcctctcagcctctgagcctgcgcccagaggcctgtcggcccgcagcaggaggagcagtgcacaccagaggcctggatttcgcctgcgacatctacatctgggcaccactggccggcacatgtggcgtgctgctgctgagcctggtcatcaccctgtactgcaagagaggcaggaagaagctgctgtatatcttcaagcagcccttcatgcggcccgtgcagacaacccaggaggaggatggctgcagctgtaggttcccagaggaggaggagggcggctgtgagctgagagtgaagttttccaggtctgccgacgcaccagcataccagcagggacagaaccagctgtataacgagctgaatctgggccggagagaggagtacgatgtgctggacaagaggcggggccgggaccccgagatgggaggcaagcctcggagaaagaacccacaggagggcctgtacaatgagctgcagaaggataagatggccgaggcctatagcgagatcggcatgaagggagagaggcgccggggcaagggacacgacggcctgtatcagggcctgtcaaccgctaccaaagacacctacgacgctctgcacatgcaggctctgcccccccgc

SEQ ID NO: 97 - DNA, 294 bp, Homo sapiens
  source 1..294: mol_type = other DNA
  misc_feature 1..294: note = truncated BCMA fragment
atgttgcagatggctgggcagtgctcccaaaatgaatattttgacagtttgttgcatgcttgcataccttgtcaacttcgatgttcttctaatactcctcctctaacatgtcagcgttattgtaatgcaagtgtgaccaattcagtgaaaggaacgaatgcgattctctggacctgtttgggactgagcttaataatttctttggcagttttcgtgctaatgtttttgctaaggaagataaactctgaaccattaaaggacgagtttaaaaacacaggatcaggtctcctgggc